European Patent Application EP 4 130 281 A1, published February 8, 2023. Title: Microorganism having increased glycine productivity and method for producing fermented composition using the same. Applicant: CJ CheilJedang Corporation. The sequence listing filed with the application follows.

SEQUENCE LISTING (18 sequences)

SEQ ID NO: 1 - DNA, 65 bp, Corynebacterium glutamicum
aattattcgactaatatcctcccccaaacacacattgataactgttgtgtggaagaatgtaccga

SEQ ID NO: 2 - DNA, 65 bp, Artificial Sequence
  hisEG promoter
aattattcgactaatatcctcccccaaacacacattgataactgttgtgtggtataatgtaccga

SEQ ID NO: 3 - DNA, 65 bp, Artificial Sequence
  hisEG promoter
aattattcgactaatatcctcccccaaacacacattgataactgttgtgtggtataatggaccga

SEQ ID NO: 4 - protein, 281 aa, Corynebacterium glutamicum [sequence omitted]

SEQ ID NO: 5 - protein, 281 aa, Artificial Sequence
  HisG(G233H)
MLKIAVPNKGSLSERAMEILAEAGYAGRGDSKSLNVFDEANNVEFFFLRPKDIAIYVAGGQLDLGITGRDLARDSQADVHEVLSLGFGSSTFRYAAPADEEWSIEKLDGKRIATSYPNLVRDDLAARGLSAEVLRLDGAVEVSIKLGVADAIADVVSTGRTLRQQGLAPFGEVLCTSEAVIVGRKDEKVTPEQQILLRRIQGILHAQNFLMLDYNVDRDNLDAATAVTPGLSHPTVSPLARDNWVAVRAMVPRRSANAIMDKLAGLGAEAILASEIRIARI

SEQ ID NO: 6 - protein, 281 aa, Artificial Sequence
  HisG(G233H/T235Q)
MLKIAVPNKGSLSERAMEILAEAGYAGRGDSKSLNVFDEANNVEFFFLRPKDIAIYVAGGQLDLGITGRDLARDSQADVHEVLSLGFGSSTFRYAAPADEEWSIEKLDGKRIATSYPNLVRDDLAARGLSAEVLRLDGAVEVSIKLGVADAIADVVSTGRTLRQQGLAPFGEVLCTSEAVIVGRKDEKVTPEQQILLRRIQGILHAQNFLMLDYNVDRDNLDAATAVTPGLSHPQVSPLARDNWVAVRAMVPRRSANAIMDKLAGLGAEAILASEIRIARI

SEQ ID NO: 7 - DNA, 33 bp, Artificial Sequence
  hisEG-pro-2mt-AF
gatcctctagagtcgacttcgacgaatccctcg

SEQ ID NO: 8 - DNA, 32 bp, Artificial Sequence
  hisEG-pro-2mt-AR
cggtacattataccacacaacagttatcaatg

SEQ ID NO: 9 - DNA, 32 bp, Artificial Sequence
  hisEG-pro-2mt-BF
gtggtataatgtaccgagtgaagacatttgac

SEQ ID NO: 10 - DNA, 32 bp, Artificial Sequence
  hisEG-pro-2mt-BR
atgcctgcaggtcgactgatacccaaatcgag

SEQ ID NO: 11 - DNA, 32 bp, Artificial Sequence
  hisEG-pro-3mt-AR
cggtccattataccacacaacagttatcaatg

SEQ ID NO: 12 - DNA, 32 bp, Artificial Sequence
  hisEG-pro-3mt-BF
gtggtataatggaccgagtgaagacatttgac

SEQ ID NO: 13 - DNA, 34 bp, Artificial Sequence
  hisG(G233H)-AF
gatcctctagagtcgaccccaaacaagggctcgc

SEQ ID NO: 14 - DNA, 28 bp, Artificial Sequence
  hisG(G233H)-AR
cgtgccagtggggataccgttgggtggg

SEQ ID NO: 15 - DNA, 30 bp, Artificial Sequence
  hisG(G233H)-BF
aaccccaggcctatcccacccaacggtatc

SEQ ID NO: 16 - DNA, 33 bp, Artificial Sequence
  hisG(G233H)-BR
atgcctgcaggtcgacgcaaggttggcaacaac

SEQ ID NO: 17 - DNA, 28 bp, Artificial Sequence
  hisG(G233H/T235Q)-AR
cgtgccagtggggatacctgtgggtggg

SEQ ID NO: 18 - DNA, 30 bp, Artificial Sequence
  hisG(G233H/T235Q)-BF
aaccccaggcctatcccacccacaggtatc